European Patent Application EP 4 166 162 A1, published April 19, 2023. Title: Deoxycholic acid-Peptide Conjugate Having Anti-Obesity Activity and Uses Thereof. Applicant: CAREGEN CO., LTD. The sequence listing filed with the application follows.

SEQUENCE LISTING (31 sequences)

SEQ ID NO: 1 - protein, 5 aa, Artificial Sequence
  Peptide
KFLIK

SEQ ID NO: 2 - DNA, 20 bp, Artificial Sequence
  Forward primer for Leptin
ggatcaggttttgtggtgct

SEQ ID NO: 3 - DNA, 20 bp, Artificial Sequence
  Reverse primer for Leptin
ttgtggcccataaagtcctc

SEQ ID NO: 4 - DNA, 20 bp, Artificial Sequence
  Forward primer for Adiponectin
tcctgctttggtccctccac

SEQ ID NO: 5 - DNA, 20 bp, Artificial Sequence
  Reverse primer for Adiponectin
tctccagccccacactgaac

SEQ ID NO: 6 - DNA, 20 bp, Artificial Sequence
  Forward primer for AMPK alpha
tcaccggacataaagtggct

SEQ ID NO: 7 - DNA, 20 bp, Artificial Sequence
  Reverse primer for AMPK alpha
tgatgatgtgagggtgcctg

SEQ ID NO: 8 - DNA, 17 bp, Artificial Sequence
  Forward primer for HSL
ggacacacacacacctg

SEQ ID NO: 9 - DNA, 20 bp, Artificial Sequence
  Reverse primer for HSL
ccctttcgcagcaactttag

SEQ ID NO: 10 - DNA, 20 bp, Artificial Sequence
  Forward primer for PDE3b
tgattgacccaagccttccc

SEQ ID NO: 11 - DNA, 20 bp, Artificial Sequence
  Reverse primer for PDE3b
tcttaccactgctgcgatcc

SEQ ID NO: 12 - DNA, 21 bp, Artificial Sequence
  Forward primer for PGCLa
atgtgcagccaagactctgta

SEQ ID NO: 13 - DNA, 21 bp, Artificial Sequence
  Reverse primer for PGCLa
cgctacaccacttcaatccac

SEQ ID NO: 14 - DNA, 20 bp, Artificial Sequence
  Forward primer for PLIN
aaggatcctgcacctcacac

SEQ ID NO: 15 - DNA, 20 bp, Artificial Sequence
  Reverse primer for PLIN
cctctgctgaagggttatcg

SEQ ID NO: 16 - DNA, 24 bp, Artificial Sequence
  Forward primer for ACC alpha
accttactgccatcccatgtgcta

SEQ ID NO: 17 - DNA, 24 bp, Artificial Sequence
  Reverse primer for ACC alpha
gtgcctgatgatcgcacgaacaaa

SEQ ID NO: 18 - DNA, 19 bp, Artificial Sequence
  Forward primer for FAS
tgctggcactacagaatgc

SEQ ID NO: 19 - DNA, 20 bp, Artificial Sequence
  Reverse primer for FAS
aacagcctcagagcgacaat

SEQ ID NO: 20 - DNA, 20 bp, Artificial Sequence
  Forward primer for PPAR gamma
atgggtgaaactctgggaga

SEQ ID NO: 21 - DNA, 20 bp, Artificial Sequence
  Reverse primer for PPAR gamma
gagctgattccgaagttggt

SEQ ID NO: 22 - DNA, 20 bp, Artificial Sequence
  Forward primer for GAPDH
gtgatggcatggactgtggt

SEQ ID NO: 23 - DNA, 20 bp, Artificial Sequence
  Reverse primer for GAPDH
ggagccaaaagggtcatcat

SEQ ID NO: 24 - DNA, 20 bp, Artificial Sequence
  Forward primer for UCP1
cctgcctctctcggaaacaa

SEQ ID NO: 25 - DNA, 19 bp, Artificial Sequence
  Reverse primer for UCP1
gtagcggggtttatcccat

SEQ ID NO: 26 - DNA, 19 bp, Artificial Sequence
  Forward primer for PRDM
ccccacattccgctgtgat

SEQ ID NO: 27 - DNA, 19 bp, Artificial Sequence
  Reverse primer for PRDM
ctcgcaatccttgcactca

SEQ ID NO: 28 - DNA, 20 bp, Artificial Sequence
  Forward primer for Cidea
cgggaatagccagagtcacc

SEQ ID NO: 29 - DNA, 20 bp, Artificial Sequence
  Reverse primer for Cidea
tgtgcatcggatgtcgtagg

SEQ ID NO: 30 - DNA, 20 bp, Artificial Sequence
  Forward primer for IL-15
tgtcttcattttgggctgtg

SEQ ID NO: 31 - DNA, 20 bp, Artificial Sequence
  Reverse primer for IL-15
tgcaactgggatgaaagtca